European Patent Specification EP 3 714 064 B1, published September 18, 2024. Title: METHODS AND KITS FOR AMPLIFICATION OF APOPTOTIC CELL-FREE DNA AND OTHER SHORT DNA FRAGMENTS. Applicant: Expedeon Limited. The sequence listing filed with the application follows.

SEQUENCE LISTING (10 sequences)

SEQ ID NO: 1 - DNA, 36 bp, artificial
  Adaptor 1
taacatttgttggccactcaggccaacaaatgttat

SEQ ID NO: 2 - DNA, 39 bp, Artificial
  Adaptor 2
taacatttgttggccttcctcttggccaacaaatgttat

SEQ ID NO: 3 - DNA, 43 bp, Artificial
  Adaptor 3
taacatttgttggccttttcctcttttggccaacaaatgttat

SEQ ID NO: 4 - DNA, 51 bp, Artificial
  Adaptor 4
taacatttgttggccttttttttcctcttttttttggccaacaaatgttat

SEQ ID NO: 5 - DNA, 36 bp, Artificial; identical to SEQ ID NO: 1
  Adaptor 5

SEQ ID NO: 6 - DNA, 39 bp, Artificial; identical to SEQ ID NO: 2
  Adaptor 6

SEQ ID NO: 7 - DNA, 43 bp, Artificial; identical to SEQ ID NO: 3
  Adaptor 7

SEQ ID NO: 8 - DNA, 51 bp, Artificial; identical to SEQ ID NO: 4
  Adaptor 8

SEQ ID NO: 9 - DNA, 21 bp, Artificial
  Primer
  misc_feature (10)..(15): n is a, c, g, or t
cgactcgagnnnnnnatgtgg

SEQ ID NO: 10 - protein, 293 aa, Thermus thermophilus
MRPIEHALSYAAQGYGVLPLRPGGKEPLGKLVPHGLKNASRDPATLEAWWRSCPRCGVGILPGPEVLVLDFDDPEAWEGLRQEHPALEAAPRQRTPKGGRHVFLRLPEGVRLSASVRAIPGVDLRGMGRAYVVAAPTRLKDGRTYTWEAPLTPPEELPPVPQALLLKLLPPPPPPRPSWGAVGTASPKRLQALLQAYAAQVARTPEGQRHLTLIRYAVAAGGLIPHGLDPREAEEVLVAAAMSAGLPEWEARDAVRWGLGVGASRPLVLESSSKPPEPRTYRARVYARMRRWV